European Patent Application EP 4 663 245 A2, published December 17, 2025. Title: METHODS AND COMPOSITIONS FOR MACROPHAGE POLARIZATION. Applicant: LONZA SALES AG. Application WO PCT/US2019/017731, filed February 12, 2019. The sequence listing filed with the application follows.

SEQUENCE LISTING (6 sequences)

SEQ ID NO: 1 - DNA, 20 bp, synthetic construct
  misc_feature 1..20: note = source = /note="Description of Artificial Sequence: Synthetic oligonucleotide"
  source 1..20: mol_type = other DNA
taagctgataattcaactca

SEQ ID NO: 2 - DNA, 20 bp, synthetic construct
  misc_feature 1..20: note = source = /note="Description of Artificial Sequence: Synthetic oligonucleotide"
  source 1..20: mol_type = other DNA
tgagcgaatggacaggtctt

SEQ ID NO: 3 - DNA, 20 bp, synthetic construct
  misc_feature 1..20: note = source = /note="Description of Artificial Sequence: Synthetic oligonucleotide"
  source 1..20: mol_type = other DNA
tggatttaaaggcaggcggc

SEQ ID NO: 4 - DNA, 20 bp, synthetic construct
  misc_feature 1..20: note = source = /note="Description of Artificial Sequence: Synthetic oligonucleotide"
  source 1..20: mol_type = other DNA
ttgggtaaagtcgtgcagca

SEQ ID NO: 5 - DNA, 20 bp, synthetic construct
  misc_feature 1..20: note = source = /note="Description of Artificial Sequence: Synthetic oligonucleotide"
  source 1..20: mol_type = other DNA
gtgcagtattgtagccaggc

SEQ ID NO: 6 - DNA, 20 bp, synthetic construct
  misc_feature 1..20: note = source = /note="Description of Artificial Sequence: Synthetic oligonucleotide"
  source 1..20: mol_type = other DNA
gtagcatgtaaatatagccc